European Patent Specification EP 3 676 280 B1, published March 19, 2025. Title: Method for purifying anti-IL-6 receptor antibodies. Applicant: Fresenius Kabi Deutschland GmbH. The sequence listing filed with the application follows.

SEQUENCE LISTING (2 sequences)

SEQ ID NO: 1 - protein, 107 aa, Artificial sequence [sequence omitted]

SEQ ID NO: 2 - protein, 119 aa, Artificial sequence
  Heavy chain tocilizumab
  misc_feature (1)..(1): Xaa can be any naturally occurring amino acid
XVQLQESGPGLVRPSQTLSLTCTVSGYSITSDHAWSWVRQPPGRGLEWIGYISYSGITTYNPSLKSRVTMLRDTSKNQFSLRLSSVTAADTAVYYCARSLARTTAMDYWGQGSLVTVSS